European Patent Application EP 4 219 533 A1, published August 2, 2023. Title: Recombinant microorganism comprising polynucleotide encoding target product binding protein fused to export signal sequence, composition comprising the same and method of producing target product using the same. Applicant: Korea Research Institute of Chemical Technology. The sequence listing filed with the application follows.

SEQUENCE LISTING (36 sequences)

SEQ ID NO: 1 - protein, 403 aa, Homo sapiens
MSGRVGDLSPRQKEALAKFRENVQDVLPALPNPDDYFLLRWLRARSFDLQKSEAMLRKHVEFRKQKDIDNIISWQPPEVIQQYLSGGMCGYDLDGCPVWYDIIGPLDAKGLLFSASKQDLLRTKMRECELLLQECAHQTTKLGRKVETITIIYDCEGLGLKHLWKPAVEAYGEFLCMFEENYPETLKRLFVVKAPKLFPVAYNLIKPFLSEDTRKKIMVLGANWKEVLLKHISPDQVPVEYGGTMTDPDGNPKCKSKINYGGDIPRKYYVRDQVKQQYEHSVQISRGSSHQVEYEILFPGCVLRWQFMSDGADVGFGIFLKTKMGERQRAGEMTEVLPNQRYNSHLVPEDGTLTCSDPGIYVLRFDNTYSFIHAKKVNFTVEVLLPDKASEEKMKQLGAGTPK

SEQ ID NO: 2 - protein, 275 aa, Artificial
  truncated SPF
MSGRVGDLSPRQKEALAKFRENVQDVLPALPNPDDYFLLRWLRARSFDLQKSEAMLRKHVEFRKQKDIDNIISWQPPEVIQQYLSGGMCGYDLDGCPVWYDIIGPLDAKGLLFSASKQDLLRTKMRECELLLQECAHQTTKLGRKVETITIIYDCEGLGLKHLWKPAVEAYGEFLCMFEENYPETLKRLFVVKAPKLFPVAYNLIKPFLSEDTRKKIMVLGANWKEVLLKHISPDQVPVEYGGTMTDPDGNPKCKSKINYGGDIPRKYYVRDQVK

SEQ ID NO: 3 - DNA, 1209 bp, Homo sapiens
atgagcggcagagtcggcgatctgagccccaggcagaaggaggcattggccaagtttcgggagaatgtccaggatgtgctgccggccctgccgaatccagatgactattttctcctgcgttggctccgagccagaagcttcgacctgcagaagtcggaggccatgctccggaagcatgtggagttccgaaagcaaaaggacattgacaacatcattagctggcagcctccagaggtgatccaacagtatctgtcagggggtatgtgtggctatgacctggatggctgcccagtctggtacgacataattggacctctggatgccaagggtctgctgttctcagcctccaaacaggacctgctgaggaccaagatgcgggagtgtgagctgcttctgcaagagtgtgcccaccagaccacaaagttggggaggaaggtggagaccatcaccataatttatgactgcgaggggcttggcctcaagcatctctggaagcctgctgtggaggcctatggagagtttctctgcatgtttgaggaaaattatcccgaaacactgaagcgtctttttgttgttaaagcccccaaactgtttcctgtggcctataacctcatcaaacccttcctgagtgaggacactcgtaagaagatcatggtcctgggagcaaattggaaggaggttttactgaaacatatcagccctgaccaggtgcctgtggagtatgggggcaccatgactgaccctgatggaaaccccaagtgcaaatccaagatcaactacgggggtgacatccccaggaagtattatgtgcgagaccaggtgaaacagcagtatgaacacagcgtgcagatttcccgtggctcctcccaccaagtggagtatgagatcctcttccctggctgtgtcctcaggtggcagtttatgtcagatggagcggatgttggttttgggattttcctgaagaccaagatgggagagaggcagcgggcaggggagatgacagaggtgctgcccaaccagaggtacaactcccacctggtccctgaagatgggaccctcacctgcagtgatcctggcatctatgtcctgcggtttgacaacacctacagcttcattcatgccaagaaggtcaatttcactgtggaggtcctgcttccagacaaagcctcagaagagaagatgaaacagctgggggcaggcaccccgaaa

SEQ ID NO: 4 - DNA, 831 bp, Artificial
  gene for tSPF
atggaattcagcggtagagttggggatttgtctcctagacaaaaagaggcgttagctaagtttagagaaaatgtacaagacgtcttaccagcccttccaaatccagatgactatttcttgctaagatggttgagagctcgaagttttgatttgcagaagtctgaggctatgcttagaaaacatgttgaatttcggaagcaaaaagatattgataacatcatatcatggcaaccaccagaagtgattcagcaatacttgtctggtggcatgtgtggttacgacttagacggctgcccagtttggtacgacatcatcggtccattggatgccaagggattgttgttctctgcatcaaaacaagatcttctcagaacaaaaatgcgtgaatgtgaacttttactacaagagtgtgcacaccagacaacaaaattgggtagaaaagttgaaactattaccgcaatctacgattgcgaaggcttaggattaaagcatttgtggaagcctgccgtggaagcatacggtgaagctctgtgcatgttcgaagagaattaccctgaaactctgaagagactgttcgtagtcaaagctccaaaattattcccagttgcctacaacttgattaagccattcctttccgaggacactagaaaaaagataatggtcctaggtgcaaactggaaggaagtactactcaagcatatctccccagatcaagtccctgttgagtacggtggaaccatgacagatcctgatggaaaccctaagtgtaagtcaaagattaactatgggggtgatattccacgtaagtactacgtgagagatcaagttaag

SEQ ID NO: 5 - protein, 19 aa, S.cerevisiae
MLLQAFLFLLAGFAAKISA

SEQ ID NO: 6 - protein, 17 aa, S.cerevisiae
MFKSVVYSILAASLANA

SEQ ID NO: 7 - protein, 89 aa, S.cerevisiae
MRFPSIFTAVLFAASSALAAPVNTTTEDETAQIPAEAVIGYSDLEGDFDVAVLPFSNSTNNGLLFINTTIASIAAKEEGVSLEKREAEA

SEQ ID NO: 8 - DNA, 57 bp, Artificial
  Suc2 nucleotide sequence
atgcttttgcaagctttccttttccttttggctggttttgcagccaaaatatctgca

SEQ ID NO: 9 - DNA, 51 bp, S.cerevisiae
atgtttaaatctgttgtttattcaattttagccgcttctttggccaatgca

SEQ ID NO: 10 - DNA, 266 bp, S.cerevisiae
atgagatttccttcaatttttactgcagttttattcgcagcatcctccgcattagctgctccagtcaacactacaacagaagatgaaacggcacaaattccggctgaagctgtcatcggttacttagatttagaaggggatttcgatgttgctgttttgccattttccaacagcacaaataacgggttattgtttataaatactactattgccagcattgctgctaaagaagaaggggtatctttggataaaagagaggctgaagc

SEQ ID NO: 11 - protein, 527 aa, S.cerevisiae
MAADQLVKTEVTKKSFTAPVQKASTPVLTNKTVISGSKVKSLSSAQSSSSGPSSSSEEDDSRDIESLDKKIRPLEELEALLSSGNTKQLKNKEVAALVIHGKLPLYALEKKLGDTTRAVAVRRKALSILAEAPVLASDRLPYKNYDYDRVFGACCENVIGYMPLPVGVIGPLVIDGTSYHIPMATTEGCLVASAMRGCKAINAGGGATTVLTKDGMTRGPVVRFPTLKRSGACKIWLDSEEGQNAIKKAFNSTSRFARLQHIQTCLAGDLLFMRFRTTTGDAMGMNMISKGVEYSLKQMVEEYGWEDMEVVSVSGNYCTDKKPAAINWIEGRGKSVVAEATIPGDVVRKVLKSDVSALVELNIAKNLVGSAMAGSVGGFNAHAANLVTAVFLALGQDPAQNVESSNCITLMKEVDGDLRISVSMPSIEVGTIGGGTVLEPQGAMLDLLGVRGPHATAPGTNARQLARIVACAVLAGELSLCAALAAGHLVQSHMTHNRKPAEPTKPNNLDATDINRLKDGSVTCIKS

SEQ ID NO: 12 - protein, 352 aa, S.cerevisiae
MASEKEIRRERFLNVFPKLVEELNASLLAYGMPKEACDWYAHSLNYNTPGGKLNRGLSVVDTYAILSNKTVEQLGQEEYEKVAILGWCIELLQAYFLVADDMMDKSITRRGQPCWYKVPEVGEIAINDAFMLEAAIYKLLKSHFRNEKYYIDITELFHEVTFQTELGQLMDLITAPEDKVDLSKFSLKKHSFIVTFKTAYYSFYLPVALAMYVAGITDEKDLKQARDVLIPLGEYFQIQDDYLDCFGTPEQIGKIGTDIQDNKCSWVINKALELASAEQRKTLDENYGKKDSVAEAKCKKIFNDLKIEQLYHEYEESIAKDLKAKISQVDESRGFKADVLTAFLNKVYKRSK

SEQ ID NO: 13 - protein, 224 aa, S.cerevisiae
MSVINFTGSSGPLVKVCGLQSTEAAECALDSDADLLGIICVPNRKRTIDPVIARKISSLVKAYKNSSGTPKYLVGVFRNQPKEDVLALVNDYGIDIVQLHGDESWQEYQEFLGLPVIKRLVFPKDCNILLSAASQKPHSFIPLFDSEAGGTGELLDWNSISDWVGRQESPESLHFMLAGGLTPENVGDALRLNGVIGVDVSGGVETNGVKDSNKIANFVKNAKK

SEQ ID NO: 14 - protein, 364 aa, S.cerevisiae
MSAPKKIVVLPGDHVGQEITAEAIKVLKAISDVRSNVKFDFENHLIGGAAIDATGVPLPDEALEASKKADAVLLGAVGGPKWGTGSVRPEQGLLKIRKELQLYANLRPCNFASDSLLDLSPIKPQFAKGTDFVVVRELVGGIYFGKRKEDDGDGVAWDSEQYTVPEVQRITRMAAFMALQHEPPLPIWSLDKANVLASSRLWRKTVEETIKNEFPTLKVQHQLIDSAAMILVKNPTHLNGIIITSNMFGDIISDEASVIPGSLGLLPSASLASLPDKNTAFGLYEPCHGSAPDLPKNKVNPIATILSAAMMLKLSLNLPEEGKAIEDAVKKVLDAGIRTGDLGGSNSTTEVGDAVAEEVKKILA

SEQ ID NO: 15 - protein, 220 aa, S.cerevisiae [sequence omitted]

SEQ ID NO: 16 - protein, 134 aa, S.cerevisiae
MIELDYVKGEDTIVEATSTSPWLMRSPLARAAEKRGSGLFFDINEGHGQHRDVIVAYGVSKPKRRSPHPHGNKAADKRKTTEKEPERKKRVGAPRTCKKICIQLLYRFNFTVLGIGNVCNIDLLLGTVSATNAI

SEQ ID NO: 17 - DNA, 1584 bp, S.cerevisiae
atggctgcagaccaattggtgaagactgaagtcaccaagaagtcttttactgctcctgtacaaaaggcttctacaccagttttaaccaataaaacagtcatttctggatcgaaagtcaaaagtttatcatctgcgcaatcgagctcatcaggaccttcatcatctagtgaggaagatgattcccgcgatattgaaagcttggataagaaaatacgtcctttagaagaattagaagcattattaagtagtggaaatacaaaacaattgaagaacaaagaggtcgctgccttggttattcacggtaagttacctttgtacgctttggagaaaaaattaggtgatactacgagagcggttgcggtacgtaggaaggctctttcaattttggcagaagctcctgtattagcatctgatcgtttaccatataaaaattatgactacgaccgcgtatttggcgcttgttgtgaaaatgttataggttacatgcctttgcccgttggtgttataggccccttggttatcgatggtacatcttatcatataccaatggcaactacagagggttgtttggtagcttctgccatgcgtggctgtaaggcaatcaatgctggcggtggtgcaacaactgttttaactaaggatggtatgacaagaggcccagtagtccgtttcccaactttgaaaagatctggtgcctgtaagatatggttagactcagaagagggacaaaacgcaattaaaaaagcttttaactctacatcaagatttgcacgtctgcaacatattcaaacttgtctagcaggagatttactcttcatgagatttagaacaactactggtgacgcaatgggtatgaatatgatttctaagggtgtcgaatactcattaaagcaaatggtagaagagtatggctgggaagatatggaggttgtctccgtttctggtaactactgtaccgacaaaaaaccagctgccatcaactggatcgaaggtcgtggtaagagtgtcgtcgcagaagctactattcctggtgatgttgtcagaaaagtgttaaaaagtgatgtttccgcattggttgagttgaacattgctaagaatttggttggatctgcaatggctgggtctgttggtggatttaacgcacatgcagctaatttagtgacagctgttttcttggcattaggacaagatcctgcacaaaatgtcgaaagttccaactgtataacattgatgaaagaagtggacggtgatttgagaatttccgtatccatgccatccatcgaagtaggtaccatcggtggtggtactgttctagaaccacaaggtgccatgttggacttattaggtgtaagaggcccacatgctaccgctcctggtaccaacgcacgtcaattagcaagaatagttgcctgtgccgtcttggcaggtgaattatccttatgtgctgccctagcagccggccatttggttcaaagtcatatgacccacaacaggaaacctgctgaaccaacaaaacctaacaatttggacgccactgatataaatcgtttgaaagatgggtccgtcacctgcattaaatcctaa

SEQ ID NO: 18 - DNA, 1059 bp, S.cerevisiae
atggcttcagaaaaagaaattaggagagagagattcttgaacgttttccctaaattagtagaggaattgaacgcatcgcttttggcttacggtatgcctaaggaagcatgtgactggtatgcccactcattgaactacaacactccaggcggtaagctaaatagaggtttgtccgttgtggacacgtatgctattctctccaacaagaccgttgaacaattggggcaagaagaatacgaaaaggttgccattctaggttggtgcattgagttgttgcaggcttacttcttggtcgccgatgatatgatggacaagtccattaccagaagaggccaaccatgttggtacaaggttcctgaagttggggaaattgccatcaatgacgcattcatgttagaggctgctatctacaagcttttgaaatctcacttcagaaacgaaaaatactacatagatatcaccgaattgttccatgaggtcaccttccaaaccgaattgggccaattgatggacttaatcactgcacctgaagacaaagtcgacttgagtaagttctccctaaagaagcactccttcatagttactttcaagactgcttactattctttctacttgcctgtcgcattggccatgtacgttgccggtatcacggatgaaaaggatttgaaacaagccagagatgtcttgattccattgggtgaatacttccaaattcaagatgactacttagactgcttcggtaccccagaacagatcggtaagatcggtacagatatccaagataacaaatgttcttgggtaatcaacaaggcattggaacttgcttccgcagaacaaagaaagactttagacgaaaattacggtaagaaggactcagtcgcagaagccaaatgcaaaaagattttcaatgacttgaaaattgaacagctataccacgaatatgaagagtctattgccaaggatttgaaggccaaaatttctcaggtcgatgagtctcgtggcttcaaagctgatgtcttaactgcgttcttgaacaaagtttacaagagaagcaaatag

SEQ ID NO: 19 - DNA, 675 bp, S.cerevisiae
atgtctgttattaatttcacaggtagttctggtccattggtgaaagtttgcggcttgcagagcacagaggccgcagaatgtgctctagattccgatgctgacttgctgggtattatatgtgtgcccaatagaaagagaacaattgacccggttattgcaaggaaaatttcaagtcttgtaaaagcatataaaaatagttcaggcactccgaaatacttggttggcgtgtttcgtaatcaacctaaggaggatgttttggctctggtcaatgattacggcattgatatcgtccaactgcatggagatgagtcgtggcaagaataccaagagttcctcggtttgccagttattaaaagactcgtatttccaaaagactgcaacatactactcagtgcagcttcacagaaacctcattcgtttattcccttgtttgattcagaagcaggtgggacaggtgaacttttggattggaactcgatttctgactgggttggaaggcaagagagccccgaaagcttacattttatgttagctggtggactgacgccagaaaatgttggtgatgcgcttagattaaatggcgttattggtgttgatgtaagcggaggtgtggagacaaatggtgtaaaagactctaacaaaatagcaaatttcgtcaaaaatgctaagaaatag

SEQ ID NO: 20 - DNA, 1095 bp, S.cerevisiae
atgtctgcccctaagaagatcgtcgttttgccaggtgaccacgttggtcaagaaatcacagccgaagccattaaggttcttaaagctatttctgatgttcgttccaatgtcaagttcgatttcgaaaatcatttaattggtggtgctgctatcgatgctacaggtgttccacttccagatgaggcgctggaagcctccaagaaggctgatgccgttttgttaggtgctgtgggtggtcctaaatggggtaccggtagtgttagacctgaacaaggtttactaaaaatccgtaaagaacttcaattgtacgccaacttaagaccatgtaactttgcatccgactctcttttagacttatctccaatcaagccacaatttgctaaaggtactgacttcgttgttgtcagagaattagtgggaggtatttactttggtaagagaaaggaagacgatggtgatggtgtcgcttgggatagtgaacaatacaccgttccagaagtgcaaagaatcacaagaatggccgctttcatggccctacaacatgagccaccattgcctatttggtccttggataaagctaatgttttggcctcttcaagattatggagaaaaactgtggaggaaaccatcaagaacgaattccctacattgaaggttcaacatcaattgattgattctgccgccatgatcctagttaagaacccaacccacctaaatggtattataatcaccagcaacatgtttggtgatatcatctccgatgaagcctccgttatcccaggttccttgggtttgttgccatctgcgtccttggcctctttgccagacaagaacaccgcatttggtttgtacgaaccatgccacggttctgctccagatttgccaaagaataaggtcaaccctatcgccactatcttgtctgctgcaatgatgttgaaattgtcattgaacttgcctgaagaaggtaaggccattgaagatgcagttaaaaaggttttggatgcaggtatcagaactggtgatttaggtggttccaacagtaccaccgaagtcggtgatgctgtcgccgaagaagttaagaaaatccttgcttaa

SEQ ID NO: 21 - DNA, 663 bp, S.cerevisiae
atgacagagcagaaagccctagtaaagcgtattacaaatgaaaccaagattcagattgcgatctctttaaagggtggtcccctagcgatagagcactcgatcttcccagaaaaagaggcagaagcagtagcagaacaggccacacaatcgcaagtgattaacgtccacacaggtatagggtttctggaccatatgatacatgctctggccaagcattccggctggtcgctaatcgttgagtgcattggtgacttacacatagacgaccatcacaccactgaagactgcgggattgctctcggtcaagcttttaaagaggccctaggggccgtgcgtggagtaaaaaggtttggatcaggatttgcgcctttggatgaggcactttccagagcggtggtagatctttcgaacaggccgtacgcagttgtcgaacttggtttgcaaagggagaaagtaggagatctctcttgcgagatgatcccgcattttcttgaaagctttgcagaggctagcagaattaccctccacgttgattgtctgcgaggcaagaatgatcatcaccgtagtgagagtgcgttcaaggctcttgcggttgccataagagaagccacctcgcccaatggtaccaacgatgttccctccaccaaaggtgttcttatgtag

SEQ ID NO: 22 - DNA, 405 bp, S.cerevisiae
atgatagaattggattatgtaaaaggtgaagataccattgtagaagcaaccagcacgtcgccgtggctgatgaggtctcctcttgcccgggccgcagaaaagaggggcagtggcctgtttttcgacataaatgaggggcatggccagcaccgagacgtcattgttgcatatggcgtatccaagccgaaacggcgctcgcctcatccccacgggaataaggcagccgacaaaagaaaaacgaccgaaaaggaaccagaaagaaaaaagagggtgggcgcgccgcggacgtgtaaaaagatatgcatccagcttctatatcgctttaactttaccgttttgggcatcgggaacgtatgtaacattgatctcctcttgggaacggtgagtgcaacgaatgcgatatag

SEQ ID NO: 23 - protein, 296 aa, Artificial
  Suc2-tSPF
MLLQAFLFLLAGFAAKISAMEFSGRVGDLSPRQKEALAKFRENVQDVLPALPNPDDYFLLRWLRARSFDLQKSEAMLRKHVEFRKQKDIDNIISWQPPEVIQQYLSGGMCGYDLDGCPVWYDIIGPLDAKGLLFSASKQDLLRTKMRECELLLQECAHQTTKLGRKVETITAIYDCEGLGLKHLWKPAVEAYGEALCMFEENYPETLKRLFVVKAPKLFPVAYNLIKPFLSEDTRKKIMVLGANWKEVLLKHISPDQVPVEYGGTMTDPDGNPKCKSKINYGGDIPRKYYVRDQVK

SEQ ID NO: 24 - protein, 294 aa, Artificial
  Pho5-SPF
MFKSVVYSILAASLANAMEFSGRVGDLSPRQKEALAKFRENVQDVLPALPNPDDYFLLRWLRARSFDLQKSEAMLRKHVEFRKQKDIDNIISWQPPEVIQQYLSGGMCGYDLDGCPVWYDIIGPLDAKGLLFSASKQDLLRTKMRECELLLQECAHQTTKLGRKVETITAIYDCEGLGLKHLWKPAVEAYGEALCMFEENYPETLKRLFVVKAPKLFPVAYNLIKPFLSEDTRKKIMVLGANWKEVLLKHISPDQVPVEYGGTMTDPDGNPKCKSKINYGGDIPRKYYVRDQVK

SEQ ID NO: 25 - protein, 366 aa, Artificial
  MFα-tSPF
MRFPSIFTAVLFAASSALAAPVNTTTEDETAQIPAEAVIGYSDLEGDFDVAVLPFSNSTNNGLLFINTTIASIAAKEEGVSLEKREAEAMEFSGRVGDLSPRQKEALAKFRENVQDVLPALPNPDDYFLLRWLRARSFDLQKSEAMLRKHVEFRKQKDIDNIISWQPPEVIQQYLSGGMCGYDLDGCPVWYDIIGPLDAKGLLFSASKQDLLRTKMRECELLLQECAHQTTKLGRKVETITAIYDCEGLGLKHLWKPAVEAYGEALCMFEENYPETLKRLFVVKAPKLFPVAYNLIKPFLSEDTRKKIMVLGANWKEVLLKHISPDQVPVEYGGTMTDPDGNPKCKSKINYGGDIPRKYYVRDQVK

SEQ ID NO: 26 - DNA, 888 bp, Artificial
  Suc2-tSPF
atgcttttgcaagctttccttttccttttggctggttttgcagccaaaatatctgcaatggaattcagcggtagagttggggatttgtctcctagacaaaaagaggcgttagctaagtttagagaaaatgtacaagacgtcttaccagcccttccaaatccagatgactatttcttgctaagatggttgagagctcgaagttttgatttgcagaagtctgaggctatgcttagaaaacatgttgaatttcggaagcaaaaagatattgataacatcatatcatggcaaccaccagaagtgattcagcaatacttgtctggtggcatgtgtggttacgacttagacggctgcccagtttggtacgacatcatcggtccattggatgccaagggattgttgttctctgcatcaaaacaagatcttctcagaacaaaaatgcgtgaatgtgaacttttactacaagagtgtgcacaccagacaacaaaattgggtagaaaagttgaaactattaccgcaatctacgattgcgaaggcttaggattaaagcatttgtggaagcctgccgtggaagcatacggtgaagctctgtgcatgttcgaagagaattaccctgaaactctgaagagactgttcgtagtcaaagctccaaaattattcccagttgcctacaacttgattaagccattcctttccgaggacactagaaaaaagataatggtcctaggtgcaaactggaaggaagtactactcaagcatatctccccagatcaagtccctgttgagtacggtggaaccatgacagatcctgatggaaaccctaagtgtaagtcaaagattaactatgggggtgatattccacgtaagtactacgtgagagatcaagttaag

SEQ ID NO: 27 - DNA, 882 bp, Artificial
  Pho5-tSPF
atgtttaaatctgttgtttattcaattttagccgcttctttggccaatgcaatggaattcagcggtagagttggggatttgtctcctagacaaaaagaggcgttagctaagtttagagaaaatgtacaagacgtcttaccagcccttccaaatccagatgactatttcttgctaagatggttgagagctcgaagttttgatttgcagaagtctgaggctatgcttagaaaacatgttgaatttcggaagcaaaaagatattgataacatcatatcatggcaaccaccagaagtgattcagcaatacttgtctggtggcatgtgtggttacgacttagacggctgcccagtttggtacgacatcatcggtccattggatgccaagggattgttgttctctgcatcaaaacaagatcttctcagaacaaaaatgcgtgaatgtgaacttttactacaagagtgtgcacaccagacaacaaaattgggtagaaaagttgaaactattaccgcaatctacgattgcgaaggcttaggattaaagcatttgtggaagcctgccgtggaagcatacggtgaagctctgtgcatgttcgaagagaattaccctgaaactctgaagagactgttcgtagtcaaagctccaaaattattcccagttgcctacaacttgattaagccattcctttccgaggacactagaaaaaagataatggtcctaggtgcaaactggaaggaagtactactcaagcatatctccccagatcaagtccctgttgagtacggtggaaccatgacagatcctgatggaaaccctaagtgtaagtcaaagattaactatgggggtgatattccacgtaagtactacgtgagagatcaagttaag

SEQ ID NO: 28 - DNA, 1098 bp, Artificial
  MFα-tSPF
atgagattcccatctattttcaccgctgtcttgttcgctgcctcctctgcattggctgcccctgttaacactaccactgaagacgagactgctcaaattccagctgaagcagttatcggttactctgaccttgagggtgatttcgacgtcgctgttttgcctttctctaactccactaacaacggtttgttgttcattaacaccactatcgcttccattgctgctaaggaagagggtgtctctctcgagaaaagagaggccgaagctatggaattcagcggtagagttggggatttgtctcctagacaaaaagaggcgttagctaagtttagagaaaatgtacaagacgtcttaccagcccttccaaatccagatgactatttcttgctaagatggttgagagctcgaagttttgatttgcagaagtctgaggctatgcttagaaaacatgttgaatttcggaagcaaaaagatattgataacatcatatcatggcaaccaccagaagtgattcagcaatacttgtctggtggcatgtgtggttacgacttagacggctgcccagtttggtacgacatcatcggtccattggatgccaagggattgttgttctctgcatcaaaacaagatcttctcagaacaaaaatgcgtgaatgtgaacttttactacaagagtgtgcacaccagacaacaaaattgggtagaaaagttgaaactattaccgcaatctacgattgcgaaggcttaggattaaagcatttgtggaagcctgccgtggaagcatacggtgaagctctgtgcatgttcgaagagaattaccctgaaactctgaagagactgttcgtagtcaaagctccaaaattattcccagttgcctacaacttgattaagccattcctttccgaggacactagaaaaaagataatggtcctaggtgcaaactggaaggaagtactactcaagcatatctccccagatcaagtccctgttgagtacggtggaaccatgacagatcctgatggaaaccctaagtgtaagtcaaagattaactatgggggtgatattccacgtaagtactacgtgagagatcaagttaag

SEQ ID NO: 29 - DNA, 6352 bp, Artificial
  p426-TEF1
aagggaacaaaagctggagctcatagcttcaaaatgtttctactccttttttactcttccagattttctcggactccgcgcatcgccgtaccacttcaaaacacccaagcacagcatactaaatttcccctctttcttcctctagggtgtcgttaattacccgtactaaaggtttggaaaagaaaaaagagaccgcctcgtttctttttcttcgtcgaaaaaggcaataaaaatttttatcacgtttctttttcttgaaaattttttttttgatttttttctctttcgatgacctcccattgatatttaagttaataaacggtcttcaatttctcaagtttcagtttcatttttcttgttctattacaactttttttacttcttgctcattagaaagaaagcatagcaatctaatctaagttttctagaactagtggatcccccgggctgcaggaattcgatatcaagcttatcgataccgtcgacctcgagtcatgtaattagttatgtcacgcttacattcacgccctccccccacatccgctctaaccgaaaaggaaggagttagacaacctgaagtctaggtccctatttatttttttatagttatgttagtattaagaacgttatttatatttcaaatttttcttttttttctgtacagacgcgtgtacgcatgtaacattatactgaaaaccttgcttgagaaggttttgggacgctcgaaggctttaatttgcggccggtacccaattcgccctatagtgagtcgtattacgcgcgctcactggccgtcgttttacaacgtcgtgactgggaaaaccctggcgttacccaacttaatcgccttgcagcacatccccctttcgccagctggcgtaatagcgaagaggcccgcaccgatcgcccttcccaacagttgcgcagcctgaatggcgaatggcgcgacgcgccctgtagcggcgcattaagcgcggcgggtgtggtggttacgcgcagcgtgaccgctacacttgccagcgccctagcgcccgctcctttcgctttcttcccttcctttctcgccacgttcgccggctttccccgtcaagctctaaatcgggggctccctttagggttccgatttagtgctttacggcacctcgaccccaaaaaacttgattagggtgatggttcacgtagtgggccatcgccctgatagacggtttttcgccctttgacgttggagtccacgttctttaatagtggactcttgttccaaactggaacaacactcaaccctatctcggtctattcttttgatttataagggattttgccgatttcggcctattggttaaaaaatgagctgatttaacaaaaatttaacgcgaattttaacaaaatattaacgtttacaatttcctgatgcggtattttctccttacgcatctgtgcggtatttcacaccgcatagggtaataactgatataattaaattgaagctctaatttgtgagtttagtatacatgcatttacttataatacagttttttagttttgctggccgcatcttctcaaatatgcttcccagcctgcttttctgtaacgttcaccctctaccttagcatcccttccctttgcaaatagtcctcttccaacaataataatgtcagatcctgtagagaccacatcatccacggttctatactgttgacccaatgcgtctcccttgtcatctaaacccacaccgggtgtcataatcaaccaatcgtaaccttcatctcttccacccatgtctctttgagcaataaagccgataacaaaatctttgtcgctcttcgcaatgtcaacagtacccttagtatattctccagtagatagggagcccttgcatgacaattctgctaacatcaaaaggcctctaggttcctttgttacttcttctgccgcctgcttcaaaccgctaacaatacctgggcccaccacaccgtgtgcattcgtaatgtctgcccattctgctattctgtatacacccgcagagtactgcaatttgactgtattaccaatgtcagcaaattttctgtcttcgaagagtaaaaaattgtacttggcggataatgcctttagcggcttaactgtgccctccatggaaaaatcagtcaagatatccacatgtgtttttagtaaacaaattttgggacctaatgcttcaactaactccagtaattccttggtggtacgaacatccaatgaagcacacaagtttgtttgcttttcgtgcatgatattaaatagcttggcagcaacaggactaggatgagtagcagcacgttccttatatgtagctttcgacatgatttatcttcgtttcctgcaggtttttgttctgtgcagttgggttaagaatactgggcaatttcatgtttcttcaacactacatatgcgtatatataccaatctaagtctgtgctccttccttcgttcttccttctgttcggagattaccgaatcaaaaaaatttcaaagaaaccgaaatcaaaaaaaagaataaaaaaaaaatgatgaattgaattgaaaagctgtggtatggtgcactctcagtacaatctgctctgatgccgcatagttaagccagccccgacacccgccaacacccgctgacgcgccctgacgggcttgtctgctcccggcatccgcttacagacaagctgtgaccgtctccgggagctgcatgtgtcagaggttttcaccgtcatcaccgaaacgcgcgagacgaaagggcctcgtgatacgcctatttttataggttaatgtcatgataataatggtttcttagtatgatccaatatcaaaggaaatgatagcattgaaggatgagactaatccaattgaggagtggcagcatatagaacagctaaagggtagtgctgaaggaagcatacgataccccgcatggaatgggataatatcacaggaggtactagactacctttcatcctacataaatagacgcatataagtacgcatttaagcataaacacgcactatgccgttcttctcatgtatatatatatacaggcaacacgcagatataggtgcgacgtgaacagtgagctgtatgtgcgcagctcgcgttgcattttcggaagcgctcgttttcggaaacgctttgaagttcctattccgaagttcctattctctagaaagtataggaacttcagagcgcttttgaaaaccaaaagcgctctgaagacgcactttcaaaaaaccaaaaacgcaccggactgtaacgagctactaaaatattgcgaataccgcttccacaaacattgctcaaaagtatctctttgctatatatctctgtgctatatccctatataacctacccatccacctttcgctccttgaacttgcatctaaactcgacctctacattttttatgtttatctctagtattactctttagacaaaaaaattgtagtaagaactattcatagagtgaatcgaaaacaatacgaaaatgtaaacatttcctatacgtagtatatagagacaaaatagaagaaaccgttcataattttctgaccaatgaagaatcatcaacgctatcactttctgttcacaaagtatgcgcaatccacatcggtatagaatataatcggggatgcctttatcttgaaaaaatgcacccgcagcttcgctagtaatcagtaaacgcgggaagtggagtcaggctttttttatggaagagaaaatagacaccaaagtagccttcttctaaccttaacggacctacagtgcaaaaagttatcaagagactgcattatagagcgcacaaaggagaaaaaaagtaatctaagatgctttgttagaaaaatagcgctctcgggatgcatttttgtagaacaaaaaagaagtatagattctttgttggtaaaatagcgctctcgcgttgcatttctgttctgtaaaaatgcagctcagattctttgtttgaaaaattagcgctctcgcgttgcatttttgttttacaaaaatgaagcacagattcttcgttggtaaaatagcgctttcgcgttgcatttctgttctgtaaaaatgcagctcagattctttgtttgaaaaattagcgctctcgcgttgcatttttgttctacaaaatgaagcacagatgcttcgttcaggtggcacttttcggggaaatgtgcgcggaacccctatttgtttatttttctaaatacattcaaatatgtatccgctcatgagacaataaccctgataaatgcttcaataatattgaaaaaggaagagtatgagtattcaacatttccgtgtcgcccttattcccttttttgcggcattttgccttcctgtttttgctcacccagaaacgctggtgaaagtaaaagatgctgaagatcagttgggtgcacgagtgggttacatcgaactggatctcaacagcggtaagatccttgagagttttcgccccgaagaacgttttccaatgatgagcacttttaaagttctgctatgtggcgcggtattatcccgtattgacgccgggcaagagcaactcggtcgccgcatacactattctcagaatgacttggttgagtactcaccagtcacagaaaagcatcttacggatggcatgacagtaagagaattatgcagtgctgccataaccatgagtgataacactgcggccaacttacttctgacaacgatcggaggaccgaaggagctaaccgcttttttgcacaacatgggggatcatgtaactcgccttgatcgttgggaaccggagctgaatgaagccataccaaacgacgagcgtgacaccacgatgcctgtagcaatggcaacaacgttgcgcaaactattaactggcgaactacttactctagcttcccggcaacaattaatagactggatggaggcggataaagttgcaggaccacttctgcgctcggcccttccggctggctggtttattgctgataaatctggagccggtgagcgtgggtctcgcggtatcattgcagcactggggccagatggtaagccctcccgtatcgtagttatctacacgacggggagtcaggcaactatggatgaacgaaatagacagatcgctgagataggtgcctcactgattaagcattggtaactgtcagaccaagtttactcatatatactttagattgatttaaaacttcatttttaatttaaaaggatctaggtgaagatcctttttgataatctcatgaccaaaatcccttaacgtgagttttcgttccactgagcgtcagaccccgtagaaaagatcaaaggatcttcttgagatcctttttttctgcgcgtaatctgctgcttgcaaacaaaaaaaccaccgctaccagcggtggtttgtttgccggatcaagagctaccaactctttttccgaaggtaactggcttcagcagagcgcagataccaaatactgtccttctagtgtagccgtagttaggccaccacttcaagaactctgtagcaccgcctacatacctcgctctgctaatcctgttaccagtggctgctgccagtggcgataagtcgtgtcttaccgggttggactcaagacgatagttaccggataaggcgcagcggtcgggctgaacggggggttcgtgcacacagcccagcttggagcgaacgacctacaccgaactgagatacctacagcgtgagctatgagaaagcgccacgcttcccgaagggagaaaggcggacaggtatccggtaagcggcagggtcggaacaggagagcgcacgagggagcttccagggggaaacgcctggtatctttatagtcctgtcgggtttcgccacctctgacttgagcgtcgatttttgtgatgctcgtcaggggggcggagcctatggaaaaacgccagcaacgcggcctttttacggttcctggccttttgctggccttttgctcacatgttctttcctgcgttatcccctgattctgtggataaccgtattaccgcctttgagtgagctgataccgctcgccgcagccgaacgaccgagcgcagcgagtcagtgagcgaggaagcggaagagcgcccaatacgcaaaccgcctctccccgcgcgttggccgattcattaatgcagctggcacgacaggtttcccgactggaaagcgggcagtgagcgcaacgcaattaatgtgagttacctcactcattaggcaccccaggctttacactttatgcttccggctcctatgttgtgtggaattgtgagcggataacaatttcacacaggaaacagctatgaccatgattacgccaagcgcgcaattaaccctcacta

SEQ ID NO: 30 - DNA, 6270 bp, Artificial
  p415-GPD
gacgaaagggcctcgtgatacgcctatttttataggttaatgtcatgataataatggtttcttaggacggatcgcttgcctgtaacttacacgcgcctcgtatcttttaatgatggaataatttgggaatttactctgtgtttatttatttttatgttttgtatttggattttagaaagtaaataaagaaggtagaagagttacggaatgaagaaaaaaaaataaacaaaggtttaaaaaatttcaacaaaaagcgtactttacatatatatttattagacaagaaaagcagattaaatagatatacattcgattaacgataagtaaaatgtaaaatcacaggattttcgtgtgtggtcttctacacagacaagatgaaacaattcggcattaatacctgagagcaggaagagcaagataaaaggtagtatttgttggcgatccccctagagtcttttacatcttcggaaaacaaaaactattttttctttaatttctttttttactttctatttttaatttatatatttatattaaaaaatttaaattataattatttttatagcacgtgatgaaaaggacccaggtggcacttttcggggaaatgtgcgcggaacccctatttgtttatttttctaaatacattcaaatatgtatccgctcatgagacaataaccctgataaatgcttcaataatattgaaaaaggaagagtatgagtattcaacatttccgtgtcgcccttattcccttttttgcggcattttgccttcctgtttttgctcacccagaaacgctggtgaaagtaaaagatgctgaagatcagttgggtgcacgagtgggttacatcgaactggatctcaacagcggtaagatccttgagagttttcgccccgaagaacgttttccaatgatgagcacttttaaagttctgctatgtggcgcggtattatcccgtattgacgccgggcaagagcaactcggtcgccgcatacactattctcagaatgacttggttgagtactcaccagtcacagaaaagcatcttacggatggcatgacagtaagagaattatgcagtgctgccataaccatgagtgataacactgcggccaacttacttctgacaacgatcggaggaccgaaggagctaaccgcttttttgcacaacatgggggatcatgtaactcgccttgatcgttgggaaccggagctgaatgaagccataccaaacgacgagcgtgacaccacgatgcctgtagcaatggcaacaacgttgcgcaaactattaactggcgaactacttactctagcttcccggcaacaattaatagactggatggaggcggataaagttgcaggaccacttctgcgctcggcccttccggctggctggtttattgctgataaatctggagccggtgagcgtgggtctcgcggtatcattgcagcactggggccagatggtaagccctcccgtatcgtagttatctacacgacggggagtcaggcaactatggatgaacgaaatagacagatcgctgagataggtgcctcactgattaagcattggtaactgtcagaccaagtttactcatatatactttagattgatttaaaacttcatttttaatttaaaaggatctaggtgaagatcctttttgataatctcatgaccaaaatcccttaacgtgagttttcgttccactgagcgtcagaccccgtagaaaagatcaaaggatcttcttgagatcctttttttctgcgcgtaatctgctgcttgcaaacaaaaaaaccaccgctaccagcggtggtttgtttgccggatcaagagctaccaactctttttccgaaggtaactggcttcagcagagcgcagataccaaatactgtccttctagtgtagccgtagttaggccaccacttcaagaactctgtagcaccgcctacatacctcgctctgctaatcctgttaccagtggctgctgccagtggcgataagtcgtgtcttaccgggttggactcaagacgatagttaccggataaggcgcagcggtcgggctgaacggggggttcgtgcacacagcccagcttggagcgaacgacctacaccgaactgagatacctacagcgtgagctatgagaaagcgccacgcttcccgaagggagaaaggcggacaggtatccggtaagcggcagggtcggaacaggagagcgcacgagggagcttccagggggaaacgcctggtatctttatagtcctgtcgggtttcgccacctctgacttgagcgtcgatttttgtgatgctcgtcaggggggcggagcctatggaaaaacgccagcaacgcggcctttttacggttcctggccttttgctggccttttgctcacatgttctttcctgcgttatcccctgattctgtggataaccgtattaccgcctttgagtgagctgataccgctcgccgcagccgaacgaccgagcgcagcgagtcagtgagcgaggaagcggaagagcgcccaatacgcaaaccgcctctccccgcgcgttggccgattcattaatgcagctggcacgacaggtttcccgactggaaagcgggcagtgagcgcaacgcaattaatgtgagttacctcactcattaggcaccccaggctttacactttatgcttccggctcctatgttgtgtggaattgtgagcggataacaatttcacacaggaaacagctatgaccatgattacgccaagcgcgcaattaaccctcactaaagggaacaaaagctggagctcagtttatcattatcaatactcgccatttcaaagaatacgtaaataattaatagtagtgattttcctaactttatttagtcaaaaaattagccttttaattctgctgtaacccgtacatgcccaaaatagggggcgggttacacagaatatataacatcgtaggtgtctgggtgaacagtttattcctggcatccactaaatataatggagcccgctttttaagctggcatccagaaaaaaaaagaatcccagcaccaaaatattgttttcttcaccaaccatcagttcataggtccattctcttagcgcaactacagagaacaggggcacaaacaggcaaaaaacgggcacaacctcaatggagtgatgcaacctgcctggagtaaatgatgacacaaggcaattgacccacgcatgtatctatctcattttcttacaccttctattaccttctgctctctctgatttggaaaaagctgaaaaaaaaggttgaaaccagttccctgaaattattcccctacttgactaataagtatataaagacggtaggtattgattgtaattctgtaaatctatttcttaaacttcttaaattctacttttatagttagtcttttttttagttttaaaacaccagaacttagtttcgacggattctagaactagtggatcccccgggctgcaggaattcgatatcaagcttatcgataccgtcgacctcgagtcatgtaattagttatgtcacgcttacattcacgccctccccccacatccgctctaaccgaaaaggaaggagttagacaacctgaagtctaggtccctatttatttttttatagttatgttagtattaagaacgttatttatatttcaaatttttcttttttttctgtacagacgcgtgtacgcatgtaacattatactgaaaaccttgcttgagaaggttttgggacgctcgaaggctttaatttgcggccggtacccaattcgccctatagtgagtcgtattacgcgcgctcactggccgtcgttttacaacgtcgtgactgggaaaaccctggcgttacccaacttaatcgccttgcagcacatccccctttcgccagctggcgtaatagcgaagaggcccgcaccgatcgcccttcccaacagttgcgcagcctgaatggcgaatggcgcgacgcgccctgtagcggcgcattaagcgcggcgggtgtggtggttacgcgcagcgtgaccgctacacttgccagcgccctagcgcccgctcctttcgctttcttcccttcctttctcgccacgttcgccggctttccccgtcaagctctaaatcgggggctccctttagggttccgatttagtgctttacggcacctcgaccccaaaaaacttgattagggtgatggttcacgtagtgggccatcgccctgatagacggtttttcgccctttgacgttggagtccacgttctttaatagtggactcttgttccaaactggaacaacactcaaccctatctcggtctattcttttgatttataagggattttgccgatttcggcctattggttaaaaaatgagctgatttaacaaaaatttaacgcgaattttaacaaaatattaacgtttacaatttcctgatgcggtattttctccttacgcatctgtgcggtatttcacaccgcatagggtaataactgatataattaaattgaagctctaatttgtgagtttagtatacatgcatttacttataatacagttttttaagcaaggattttcttaacttcttcggcgacagcatcaccgacttcggtggtactgttggaaccacctaaatcaccagttctgatacctgcatccaaaacctttttaactgcatcttcaatggccttaccttcttcaggcaagttcaatgacaatttcaacatcattgcagcagacaagatagtggcgatagggtcaaccttattctttggcaaatctggagcagaaccgtggcatggttcgtacaaaccaaatgcggtgttcttgtctggcaaagaggccaaggacgcagatggcaacaaacccaaggaacctgggataacggaggcttcatcggagatgatatcaccaaacatgttgctggtgattataataccatttaggtgggttgggttcttaactaggatcatggcggcagaatcaatcaattgatgttgaaccttcaatgtagggaattcgttcttgatggtttcctccacagtttttctccataatcttgaagaggccaaaacattagctttatccaaggaccaaataggcaatggtggctcatgttgtagggccatgaaagcggccattcttgtgattctttgcacttctggaacggtgtattgttcactatcccaagcgacaccatcaccatcgtcttcctttctcttaccaaagtaaatacctcccactaattctctgacaacaacgaagtcagtacctttagcaaattgtggcttgattggagataagtctaaaagagagtcggatgcaaagttacatggtcttaagttggcgtacaattgaagttctttacggatttttagtaaaccttgttcaggtctaacactaccggtaccccatttaggaccacccacagcacctaacaaaacggcatcaaccttcttggaggcttccagcgcctcatctggaagtgggacacctgtagcatcgatagcagcaccaccaattaaatgattttcgaaatcgaacttgacattggaacgaacatcagaaatagctttaagaaccttaatggcttcggctgtgatttcttgaccaacgtggtcacctggcaaaacgacgatcttcttaggggcagacataggggcagacattagaatggtatatccttgaaatatatatatatattgctgaaatgtaaaaggtaagaaaagttagaaagtaagacgattgctaaccacctattggaaaaaacaataggtccttaaataatattgtcaacttcaagtattgtgatgcaagcatttagtcatgaacgcttctctattctatatgaaaagccggttccggcctctcacctttcctttttctcccaatttttcagttgaaaaaggtatatgcgtcaggcgacctctgaaattaacaaaaaatttccagtcatcgaatttgattctgtgcgatagcgcccctgtgtgttctcgttatgttgaggaaaaaaataatggttgctaagagattcgaactcttgcatcttacgatacctgagtattcccacagttttgaaaagctgtggtatggtgcactctcagtacaatctgctctgatgccgcatagttaagccagccccgacacccgccaacacccgctgacgcgccctgacgggcttgtctgctcccggcatccgcttacagacaagctgtgaccgtctccgggagctgcatgtgtcagaggttttcaccgtcatcaccgaaacgcgcga

SEQ ID NO: 31 - protein, 582 aa, XANTHOPHYLLOMYCES DENDROHOUS
MGKEQDQDKPTAIIVGCGIGGIATAARLAKEGFQVTVFEKNDYSGGRCSLIERDGYRFDQGPSLLLLPDLFKQTFEDLGEKMEDWVDLIKCEPNYVCHFHDEETFTFSTDMALLKREVERFEGKDGFDRFLSFIQEAHRHYELAVVHVLQKNFPGFAAFLRLQFIGQILALHPFESIWTRVCRYFKTDRLRRVFSFAVMYMGQSPYSAPGTYSLLQYTELTEGIWYPRGGFWQVPNTLLQIVKRNNPSAKFNFNAPVSQVLLSPAKDRATGVRLESGEEHHADVVIVNADLVYASEHLIPDDARNKIGQLGEVKRSWWADLVGGKKLKGSCSSLSFYWSMDRIVDGLGGHNIFLAEDFKGSFDTIFEELGLPADPSFYVNVPSRIDPSAAPEGKDAIVILVPCGHIDASNPQDYNKLVARARKFVIQTLSAKLGLPDFEKMIVAEKVHDAPSWEKEFNLKDGSILGLAHNFMQVLGFRPSTRHPKYDKLFFVGASTHPGTGVPIVLAGAKLTANQVLESFDRSPAPDPNMSLSVPYGKPLKSNGTGIDSQVQLKFMDLERWVYLLVLLIGAVIARSVGVLAF

SEQ ID NO: 32 - protein, 673 aa, XANTHOPHYLLOMYCES DENDROHOUS
MTALAYYQIHLIYTLPILGLLGLLTSPILTKFDIYKISILVFIAFSATTPWDSWIIRNGAWTYPSAESGQGVFGTFLDVPYEEYAFFVIQTVITGLVYVLATRHLLPSLALPKTRSSALSLALKALIPLPIIYLFTAHPSPSPDPLVTDHYFYMRALSLLITPPTMLLAALSGEYAFDWKSGRAKSTIATIMIPTVYLIWVDYVAVGQDSWSINDEKIVGWRLGGVLPIEEAMFFLLTNLMIVLGLSACDHTQALYLLHGRTIYGNKKMPSSFPLITPPVLSLFFSSRPYSSQPKRDLELAVKLLEKKSRSFFVASAGFPSEVRERLVGLYAFCRVTDDLIDSPEVSSNPHATIDMVSDFLTLLFGPPLHPSQPDKILSSPLLPPSHPSRPTGMYPLPPPPSLSPAELVQFLTERVPVQYHFAFRLLAKLQGLIPRYPLDELLRGYTTDLIFPLSTEAVQARKTPIETTADLLDYGLCVAGSVAELLVYVSWASAPSQVPATIEEREAVLVASREMGTALQLVNIARDIKGDATEGRFYLPLSFFGLRDESKLAIPTDWTEPRPQDFDKLLSLSPSSTLPSSNASESFRFEWKTYSLPLVAYAEDLAKHSYKGIDRLPTEVQAGMRAACASYLLIGREIKVVWKGDVGERRTVAGWRRVRKVLSVVMSGWEGQ

SEQ ID NO: 33 - protein, 376 aa, XANTHOPHYLLOMYCES DENDROHOUS
MDYANILTAIPLEFTPQDDIVLLEPYHYLGKNPGKEIRSQLIEAFNYWLDVKKEDLEVIQNVVGMLHTASLLMDDVEDSSVLRRGSPVAHLIYGIPQTINTANYVYFLAYQEIFKLRPTPIPMPVIPPSSASLQSSVSSASSSSSASSENGGTSTPNSQIPFSKDTYLDKVITDEILSLHRGQGLELFWRDSLTCPSEEEYVKMVLGKTGGLFRIAVRLMMAKSECDIDFVQLVNLISIYFQIRDDYMNLQSSEYAHNKNFAEDLTEGKFSFPTIHSIHANPSSRLVINTLQKKSTSPEILHHCVNYMRTETHSFEYTQEVLNTLSGALERELGRLQGEFAEANSRMDLGDVDSEGRTGKNVKLEAILKKLADIPL

SEQ ID NO: 34 - DNA, 1749 bp, XANTHOPHYLLOMYCES DENDROHOUS
atgggaaaagaacaagatcaggataaacccacagctatcatcgtgggatgtggtatcggtggaatcgccactgccgctcgtcttgctaaagaaggtttccaggtcacggtgttcgagaagaacgactactccggaggtcgatgctctttaatcgagcgagatggttatcgattcgatcaggggcccagtttgctgctcttgccagatctcttcaagcagacattcgaagatttgggggagaagatggaagattgggtcgatctcatcaagtgtgaacccaactatgtttgccacttccacgatgaagagactttcactttttcaaccgacatggcgttgctcaagcgggaagtcgagcgttttgaaggcaaagatggatttgatcggttcttgtcgtttatccaagaagcccacagacattacgagcttgctgtcgttcacgtcctgcagaagaacttccctggcttcgcagcattcttacggctacagttcattggccaaatcctggctcttcaccccttcgagtctatctggacaagagtttgtcgatatttcaagaccgacagattacgaagagtcttctcgtttgcagtgatgtacatgggtcaaagcccatacagtgcgcccggaacatattccttgctccaatacaccgaattgaccgagggcatctggtatccgagaggaggcttttggcaggttcctaatactcttcttcagatcgtcaagcgcaacaatccctcagccaagttcaatttcaacgctccagtttcccaggttcttctctctcctgccaaggaccgagcgactggtgttcgacttgaatccggcgaggaacatcacgccgatgttgtgattgtcaatgctgacctcgtttacgcctccgagcacttgattcctgacgatgccagaaacaagattggccaactgggtgaagtcaagagaagttggtgggctgacttagttggtggaaagaagctcaagggaagttgcagtagtttgagcttctactggagcatggaccgaatcgtggacggtctgggcggacacaatatcttcttggccgaggacttcaagggatcattcgacacaatcttcgaggagttgggactcccagccgatccttccttttacgtgaacgttccctcgcgaatcgatccttctgccgctcccgaaggcaaagatgctatcgtcattcttgtgccgtgtggccatatcgacgcttcgaaccctcaagattacaacaagcttgttgctcgggcaaggaagtttgtgatccaaacgctttccgccaagcttggacttcccgactttgaaaaaatgattgtggcagagaaggttcacgatgctccctcttgggagaaagaatttaacctcaaggacggaagcatcttgggactggctcacaactttatgcaagttcttggtttcaggccgagcaccagacatcccaagtatgacaagttgttctttgtcggggcttcgactcatcccggaactggggttcccatcgtcttggctggagccaagttaactgccaaccaagttctcgaatcctttgaccgatccccagctccagatcccaatatgtcactctccgtaccatatggaaaacctctcaaatcaaatggaacgggtatcgattctcaggtccagctgaagttcatggatttggagagatgggtataccttttggtgttgttgattggggccgtgatcgctcgatccgttggtgttcttgctttctga

SEQ ID NO: 35 - DNA, 2022 bp, XANTHOPHYLLOMYCES DENDROHOUS
atgacggctctcgcatattaccagatccatctgatctatactctcccaattcttggtcttctcggcctgctcacttccccgattttgacaaaatttgacatctacaaaatatcgatcctcgtatttattgcgtttagtgcaaccacaccatgggactcatggatcatcagaaatggcgcatggacatatccatcagcggagagtggccaaggcgtgtttggaacgtttctagatgttccatatgaagagtacgctttctttgtcattcaaaccgtaatcaccggcttggtctacgtcttggcaactaggcaccttctcccatctctcgcgcttcccaagactagatcgtccgccctttctctcgcgctcaaggcgctcatccctctgcccattatctacctatttaccgctcaccccagcccatcgcccgacccgctcgtgacagatcactacttctacatgcgggcactctccttactcatcaccccacctaccatgctcttggcagcattatcaggcgaatatgctttcgattggaaaagtggccgagcaaagtcaactattgcaacaatcatgatcccgacggtgtatctgatttgggtagattatgttgctgtcggtcaagactcttggtcgatcaacgatgagaagattgtagggtggaggcttggaggtgtactacccattgaggaagctatgttcttcttactgacgaatctaatgattgttctgggtctgtctgcctgcgatcatactcaggccctatacctgctacacggtcgaactatttatggcaacaaaaagatgccatcttcatttcccctcattacaccgcctgtgctctccctgttttttagcagccgaccatactcttctcagccaaaacgtgacttggaactggcagtcaagttgttggagaaaaagagccggagcttttttgttgcctcggctggatttcctagcgaagttagggagaggctggttggactatacgcattctgccgggtgactgatgatcttatcgactctcctgaagtatcttccaacccgcatgccacaattgacatggtatccgattttcttaccctactatttgggcccccgctacacccttcgcaacctgacaagatcctttcttcgcctttacttcctccttcgcacccttcccgacccacgggaatgtatcccctcccgcctcctccttcgctctcgcctgccgagctcgttcaattccttaccgaaagggttcccgttcaataccatttcgccttcaggttgctcgctaagttgcaagggctgatccctcgatacccactcgacgaactccttagaggatacaccactgatcttatctttcccttatcgacagaggcagtccaggctcggaagacgcctatcgagacaacagctgacttgctggactatggtctatgtgtagcaggctcagtcgccgagctattggtctatgtctcttgggcaagtgcaccaagtcaggtccctgccaccatagaagaaagagaagctgtgttagtggcaagccgagagatgggaactgcccttcagttggtgaacattgctagggacattaaaggggacgcaacagaagggagattttacctaccactctcattctttggtcttcgggatgaatcaaagcttgcgatcccgactgattggacggaacctcggcctcaagatttcgacaaactcctcagtctatctccttcgtccacattaccatcttcaaacgcctcagaaagcttccggttcgaatggaagacgtactcgcttccattagtcgcctacgcagaggatcttgccaaacattcttataagggaattgaccgacttcctaccgaggttcaagcgggaatgcgagcggcttgcgcgagctacctactgatcggccgagagatcaaagtcgtttggaaaggagatgtcggagagagaaggacagttgccggatggaggagagtacggaaagtcttgagtgtggtcatgagcggatgggaagggcagtga

SEQ ID NO: 36 - DNA, 1131 bp, XANTHOPHYLLOMYCES DENDROHOUS
atggattacgcgaacatcctcacagcaattccactcgagtttactcctcaggatgatatcgtgctccttgaaccgtatcactacctaggaaagaaccctggaaaagaaattcgatcacaactcatcgaggctttcaactattggttggatgtcaagaaggaggatctcgaggtcatccagaacgttgttggcatgctacataccgctagcttattaatggacgatgtggaggattcatcggtcctcaggcgtgggtcgcctgtggcccatctaatttacgggattccgcagacaataaacactgcaaactacgtctactttctggcttatcaagagatcttcaagcttcgcccaacaccgatacccatgcctgtaattcctccttcatctgcttcgcttcaatcatcagtctcctctgcatcctcctcctcctcggcctcgtctgaaaacgggggcacgtcaactcctaattcgcagattccgttctcgaaagatacgtatcttgataaagtgatcacagacgagatactttccctccatagagggcagggcctggagctattctggagagatagtctgacgtgtcctagcgaagaggaatatgtgaaaatggttcttggaaagacgggaggtttgttccgtatagcggtcagattgatgatggcaaagtcagaatgtgacatagactttgtccagcttgtcaacttgatctcaatatacttccagatcagggatgactatatgaaccttcagtcttctgagtatgcccataataagaattttgcagaggacctcacagaagggaaattcagttttcccactatccactcgattcatgccaacccctcatcgagactcgtcatcaatacgttgcagaagaaatcgacctctcctgagatccttcaccactgtgtaaactacatgcgcacagaaacccactcattcgaatatactcaggaagtcctcaacaccttgtcaggtgcactcgagagagaactaggaaggcttcaaggagagttcgcagaagctaactcaaggatggatcttggtgacgtagattcggaaggaagaacggggaagaacgtcaaattggaagcgatcctgaaaaagctagccgatatccctctgtga